European Patent Application EP 4 137 576 A1, published February 22, 2023. Title: Chromosomal integrating Cassette allowing inducible gene Expression for production of compounds via fermentation. Applicant: Justus-Liebig-Universität Gießen. The sequence listing filed with the application follows.

SEQUENCE LISTING (20 sequences)

SEQ ID NO: 1 - DNA, 21 bp, Escherichia coli
  Lac operator Sequence 1
ggcagtgagcgcaacgcaatt

SEQ ID NO: 2 - DNA, 20 bp, Escherichia coli
  Lac Operator Sequence 2
attgtgagcggataacaatt

SEQ ID NO: 3 - DNA, 20 bp, Artificial Sequence
  Standard sequencing primer (pUCM13-52, 5’ to 3’)
gctgcaaggcgattaagttg

SEQ ID NO: 4 - DNA, 124 bp, Rhodobacter sphaeroides
aagcttggcagtgagcgcaacgcaattaaattgttacggagcccaaaaaatccgcttgcgcccggggccgtctgctcctagaaaccgcttcaccgagacattgtgagcggataacaattctaga

SEQ ID NO: 5 - DNA, 4979 bp, Artificial Sequence
  Complete DNA sequence for ACIT
gaattcgtaatcatgtcatagctgtttcctgtgtgaaattgttatccgctcacaattccacacaacatacgagccggaagcataaagtgtaaagcctggggtgcctaatgagtgagctaactcacattaattgcgttgcgctcactgcccgctttccagtcgggaaacctgtcgtgccagctgcattaatgaatcggccaacgcgcggggagaggcggtttgcgtattgggcgctcttccgcttcctcgctcactgactcgctgcgctcggtcgttcggctgcggcgagcggtatcagctcactcaaaggcggtaatacggttatccacagaatcaggggataacgcaggaaagaacatgtgagcaaaaggccagcaaaaggccaggaaccgtaaaaaggccgcgttgctggcgtttttccataggctccgcccccctgacgagcatcacaaaaatcgacgctcaagtcagaggtggcgaaacccgacaggactataaagataccaggcgtttccccctggaagctccctcgtgcgctctcctgttccgaccctgccgcttaccggatacctgtccgcctttctcccttcgggaagcgtggcgctttctcaatgctcacgctgtaggtatctcagttcggtgtaggtcgttcgctccaagctgggctgtgtgcacgaaccccccgttcagcccgaccgctgcgccttatccggtaactatcgtcttgagtccaacccggtaagacacgacttatcgccactggcagcagccactggtaacaggattagcagagcgaggtatgtaggcggtgctacagagttcttgaagtggtggcctaactacggctacactagaaggacagtatttggtatctgcgctctgctgaagccagttaccttcggaaaaagagttggtagctcttgatccggcaaacaaaccaccgctggtagcggtggtttttttgtttgcaagcagcagattacgcgcagaaaaaaaggatctcaagaagatcctttgatcttttctacggggtctgacgctcagtggaacgaaaactcacgttaagggattttggtcatggcttttccgctgcataaccctgcttcggggtcattatagcgattttttcggtatatccatcctttttcgcacgatatacaggattttgccaaagggttcgtgtagactttccttggtgtatccaacggcgtcagcggggcaggataggtgaagtaggcccacccgcgagcgggtgttccttcttcactgtcccttattcgcacctggcggtgctcaacgggaatcctgctctgcgaggctggccggctaccgccggcgtaacagatgagggcaagcggatggctgatgaaaccaagccaaccaggaagggcagcccacctatcaaggtgtactgccttccagacgaacgaagagcgattgaggaaaaggcggcggcggccggcatgagcctgtcggcctacctgctggccgtcggccagggctacaaaatcacgggcgtcgtggactatgagcacgtccgcgagggcgtcccggaaaacgattccgaagcccaacctttcatagaaggcggcggtggaatcgaaatctcgtgatggcaggttgggcgtcgcttggtcggtcatttcgaaccccagagtcccgctcagaagaactcgtcaagaaggcgatagaaggcgatgcgctgcgaatcgggagcggcgataccgtaaagcacgaggaagcggtcagcccattcgccgccaagctcttcagcaatatcacgggtagccaacgctatgtcctgatagcggtccgccacacccagccggccacagtcgatgaatccagaaaagcggccattttccaccatgatattcggcaagcaggcatcgccatgggtcacgacgagatcctcgccgtcgggcatccgcgccttgagcctggcgaacagttcggctggcgcgagcccctgatgctcttcgtccagatcatcctgatcgacaagaccggcttccatccgagtacgtgctcgctcgatgcgatgtttcgcttggtggtcgaatgggcaggtagccggatcaagcgtatgcagccgccgcattgcatcagccatgatggatactttctcggcaggagcaaggtgagatgacaggagatcctgccccggcacttcgcccaatagcagccagtcccttcccgcttcagtgacaacgtcgagcacagctgcgcaaggaacgcccgtcgtggccagccacgatagccgcgctgcctcgtcttggagttcattcagggcaccggacaggtcggtcttgacaaaaagaaccgggcgcccctgcgctgacagccggaacacggcggcatcagagcagccgattgtctgttgtgcccagtcatagccgaatagcctctccacccaagcggccggagaacctgcgtgcaatccatcttgttcaatcatgcgaaacgatcctcatcctgtctcttgatcagatcttgatcccctgcgccatcagatccttggcggcaagaaagccatccagtttactttgcagggcttcccaaccttaccagagggcgccccagctggcaattccggttcgcttgctgtccataaaaccgcccagtctagctatcgccatgtaagcccactgcaagctacctgctttctctttgcgcttgcgttttcccttgtccagatagcccagtagctgacattcatccggggtcagcaccgtttctgcggactggctttctacgtgttccgcttcctttagcagcccttgcgccctgagtgcttgcggcagcgtgaagctagcttatcgcgccattcgccattcaggctgcgcaactgttgggaagggcgatcggtgcgggcctcttcgctattacgccagctggcgaaagggggatgtgctgcaaggcgattaagttgggtaacgccagggttttcccagtcacgacgttgtaaaacgacggccagtgccaagcttggcagtgagcgcaacgcaattaaattgttacggagcccaaaaaatccgcttgcgcccggggccgtctgctcctagaaaccgcttcaccgagacattgtgagcggataacaattctagacatacacaggggggacaagtcaatatggcaaccgaagagcagtctccgggttccggccgtgacgctcagttcgagcgtctgaacgcgaatctcacccgcatcgacgagctgtcgaaacggctgacggccgctctcacgaagcgcaaactgtcggaccccgcgctgcacgggccctcgggcgacgtcttcctgaaggcgatgacggcctacatggccgagatgatgcagaacccggccaagatcctcgagcatcagatcagtttctggggcaagagcctgaaacattacgtcgaggctcagcaccagctggtgaagggcgagctgaagccgccgccggacgtgacgccgaaggaccgccgcttctcgaacccgctctggcagacgcatcccttcttcaactatctcggtaccatgctgcagcgcgtacaggaaacacagaaaaaagcccgcacctgacagtgcgggctttttttttcgaccaaaggtaacgaggtaacaaccatgcgagtgttgaagtggcagaactgctgaacgcaggtctgggcggttctgataacgagtaatcgttaatccgcaaataacgtaaaaacccgcttcggcgggtttttttatggggggagtttagggaaagtcgacgcaacgcaaggcgtttcgggccaggtgcgaaaaaatgctgcggtgcagaatgagcggttgattttctgcggcgcagcatttatatccttgtcacaggataaccgggcatgagcccgctcgcaggagagagctcaggagacaaggcaatgaaaccagtaacgttatacgatgtcgcagagtatgccggtgtctcttatcagaccgtttcccgcgtggtgaaccaggccagccacgtttctgcgaaaacgcgggaaaaagtggaagcggcgatggcggagctgaattacattcccaaccgcgtggcacaacaactggcgggcaaacagtcgttgctgattggcgttgccacctccagtctggccctgcacgcgccgtcgcaaattgtcgcggcgattaaatctcgcgccgatcaactgggtgccagcgtggtggtgtcgatggtagaacgaagcggcgtcgaagcctgtaaagcggcggtgcacaatcttctcgcgcaacgcgtcagtgggctgatcattaactatccgctggatgaccaggatgccattgctgtggaagctgcctgcactaatgttccggcgttatttcttgatgtctctgaccagacacccatcaacagtattattttctcccatgaagacggtacgcgactgggcgtggagcatctggtcgcattgggtcaccagcaaatcgcgctgttagcgggcccattaagttctgtctcggcgcgtctgcgtctggctggctggcataaatatctcactcgcaatcaaattcagccgatagcggaacgggaaggcgactggagtgccatgtccggttttcaacaaaccatgcaaatgctgaatgagggcatcgttcccactgcgatgctggttgccaacgatcagatggcgctgggcgcaatgcgcgccattaccgagtccgggctgcgcgttggtgcggatatctcggtagtgggatacgacgataccgaagacagctcatgttatatcccgccgttaaccaccatcaaacaggattttcgcctgctggggcaaaccagcgtggaccgcttgctgcaactctctcagggccaggcggtgaagggcaatcagctgttgcccgtctcactggtgaaaagaaaaaccaccctggcgcccaatacgcaaaccgcctctccccgcgcgttggccgattcattaatgcagctggcacgacaggtttcccgactggaaagcgggcagtgagaattc

SEQ ID NO: 6 - DNA, 120 bp, Artificial Sequence
  sequence of the cerI promoter
gtcgaccctgccccagaggaccgaaattcaaccggaaattgccaaaggaagccttccggctacgggattcccctcatagccgaaacgggtcgggatgcgcaactatagccgtatgagctc

SEQ ID NO: 7 - DNA, 2978 bp, Artificial Sequence
  publically available cloning vector Pk18mob2
gtaatcatgtcatagctgtttcctgtgtgaaattgttatccgctcacaattccacacaacatacgagccggaagcataaagtgtaaagcctggggtgcctaatgagtgagctaactcacattaattgcgttgcgctcactgcccgctttccagtcgggaaacctgtcgtgccagctgcattaatgaatcggccaacgcgcggggagaggcggtttgcgtattgggcgctcttccgcttcctcgctcactgactcgctgcgctcggtcgttcggctgcggcgagcggtatcagctcactcaaaggcggtaatacggttatccacagaatcaggggataacgcaggaaagaacatgtgagcaaaaggccagcaaaaggccaggaaccgtaaaaaggccgcgttgctggcgtttttccataggctccgcccccctgacgagcatcacaaaaatcgacgctcaagtcagaggtggcgaaacccgacaggactataaagataccaggcgtttccccctggaagctccctcgtgcgctctcctgttccgaccctgccgcttaccggatacctgtccgcctttctcccttcgggaagcgtggcgctttctcaatgctcacgctgtaggtatctcagttcggtgtaggtcgttcgctccaagctgggctgtgtgcacgaaccccccgttcagcccgaccgctgcgccttatccggtaactatcgtcttgagtccaacccggtaagacacgacttatcgccactggcagcagccactggtaacaggattagcagagcgaggtatgtaggcggtgctacagagttcttgaagtggtggcctaactacggctacactagaaggacagtatttggtatctgcgctctgctgaagccagttaccttcggaaaaagagttggtagctcttgatccggcaaacaaaccaccgctggtagcggtggtttttttgtttgcaagcagcagattacgcgcagaaaaaaaggatctcaagaagatcctttgatcttttctacggggtctgacgctcagtggaacgaaaactcacgttaagggattttggtcatggcttttccgctgcataaccctgcttcggggtcattatagcgattttttcggtatatccatcctttttcgcacgatatacaggattttgccaaagggttcgtgtagactttccttggtgtatccaacggcgtcagcggggcaggataggtgaagtaggcccacccgcgagcgggtgttccttcttcactgtcccttattcgcacctggcggtgctcaacgggaatcctgctctgcgaggctggccggctaccgccggcgtaacagatgagggcaagcggatggctgatgaaaccaagccaaccaggaagggcagcccacctatcaaggtgtactgccttccagacgaacgaagagcgattgaggaaaaggcggcggcggccggcatgagcctgtcggcctacctgctggccgtcggccagggctacaaaatcacgggcgtcgtggactatgagcacgtccgcgagggcgtcccggaaaacgattccgaagcccaacctttcatagaaggcggcggtggaatcgaaatctcgtgatggcaggttgggcgtcgcttggtcggtcatttcgaaccccagagtcccgctcagaagaactcgtcaagaaggcgatagaaggcgatgcgctgcgaatcgggagcggcgataccgtaaagcacgaggaagcggtcagcccattcgccgccaagctcttcagcaatatcacgggtagccaacgctatgtcctgatagcggtccgccacacccagccggccacagtcgatgaatccagaaaagcggccattttccaccatgatattcggcaagcaggcatcgccatgggtcacgacgagatcctcgccgtcgggcatccgcgccttgagcctggcgaacagttcggctggcgcgagcccctgatgctcttcgtccagatcatcctgatcgacaagaccggcttccatccgagtacgtgctcgctcgatgcgatgtttcgcttggtggtcgaatgggcaggtagccggatcaagcgtatgcagccgccgcattgcatcagccatgatggatactttctcggcaggagcaaggtgagatgacaggagatcctgccccggcacttcgcccaatagcagccagtcccttcccgcttcagtgacaacgtcgagcacagctgcgcaaggaacgcccgtcgtggccagccacgatagccgcgctgcctcgtcttggagttcattcagggcaccggacaggtcggtcttgacaaaaagaaccgggcgcccctgcgctgacagccggaacacggcggcatcagagcagccgattgtctgttgtgcccagtcatagccgaatagcctctccacccaagcggccggagaacctgcgtgcaatccatcttgttcaatcatgcgaaacgatcctcatcctgtctcttgatcagatcttgatcccctgcgccatcagatccttggcggcaagaaagccatccagtttactttgcagggcttcccaaccttaccagagggcgccccagctggcaattccggttcgcttgctgtccataaaaccgcccagtctagctatcgccatgtaagcccactgcaagctacctgctttctctttgcgcttgcgttttcccttgtccagatagcccagtagctgacattcatccggggtcagcaccgtttctgcggactggctttctacgtgttccgcttcctttagcagcccttgcgccctgagtgcttgcggcagcgtgaagctagcttatcgcgccattcgccattcaggctgcgcaactgttgggaagggcgatcggtgcgggcctcttcgctattacgccagctggcgaaagggggatgtgctgcaaggcgattaagttgggtaacgccagggttttcccagtcacgacgttgtaaaacgacggccagtgcc

SEQ ID NO: 8 - DNA, 1096 bp, Escherichia coli
  Lacl gene
aggagacaaggcaatgaaaccagtaacgttatacgatgtcgcagagtatgccggtgtctcttatcagaccgtttcccgcgtggtgaaccaggccagccacgtttctgcgaaaacgcgggaaaaagtggaagcggcgatggcggagctgaattacattcccaaccgcgtggcacaacaactggcgggcaaacagtcgttgctgattggcgttgccacctccagtctggccctgcacgcgccgtcgcaaattgtcgcggcgattaaatctcgcgccgatcaactgggtgccagcgtggtggtgtcgatggtagaacgaagcggcgtcgaagcctgtaaagcggcggtgcacaatcttctcgcgcaacgcgtcagtgggctgatcattaactatccgctggatgaccaggatgccattgctgtggaagctgcctgcactaatgttccggcgttatttcttgatgtctctgaccagacacccatcaacagtattattttctcccatgaagacggtacgcgactgggcgtggagcatctggtcgcattgggtcaccagcaaatcgcgctgttagcgggcccattaagttctgtctcggcgcgtctgcgtctggctggctggcataaatatctcactcgcaatcaaattcagccgatagcggaacgggaaggcgactggagtgccatgtccggttttcaacaaaccatgcaaatgctgaatgagggcatcgttcccactgcgatgctggttgccaacgatcagatggcgctgggcgcaatgcgcgccattaccgagtccgggctgcgcgttggtgcggatatctcggtagtgggatacgacgataccgaagacagctcatgttatatcccgccgttaaccaccatcaaacaggattttcgcctgctggggcaaaccagcgtggaccgcttgctgcaactctctcagggccaggcggtgaagggcaatcagctgttgcccgtctcactggtgaaaagaaaaaccaccctggcgcccaatacgcaaaccgcctctccccgcgcgttggccgattcattaatgcagctggcacgacaggtttcccgactggaaagcgggcagtga

SEQ ID NO: 9 - DNA, 219 bp, Escherichia coli
  tandem terminator sequence
atgctgcagcgcgtacaggaaacacagaaaaaagcccgcacctgacagtgcgggctttttttttcgaccaaaggtaacgaggtaacaaccatgcgagtgttgaagtggcagaactgctgaacgcaggtctgggcggttctgataacgagtaatcgttaatccgcaaataacgtaaaaacccgcttcggcgggtttttttatggggggagtttagggaaa

SEQ ID NO: 10 - DNA, 127 bp, Rhodobacter sphaeroides
  phaP promoter sequence
gcaacgcaaggcgtttcgggccaggtgcgaaaaaatgctgcggtgcagaatgagcggttgattttctgcggcgcagcatttatatccttgtcacaggataaccgggcatgagcccgctcgcaggaga

SEQ ID NO: 11 - DNA, 108 bp, Rhodobacter sphaeroides
  sequence for the promoter for cerI
cctgccccagaggaccgaaattcaaccggaaattgccaaaggaagccttccggctacgggattcccctcatagccgaaacgggtcgggatgcgcaactatagccgtat

SEQ ID NO: 12 - DNA, 423 bp, Sinorhizobium meliloti
ttcggtgttacggcatggctaatcaacaggctgtcctcaatttgctggatatcgtggaatatggaggttgcgcagaccccgagcgcttcttcgccctgatgcgtcgaaccttcaacatctcgcatctcctgtatctggaggcggagtctcttccggatggtttgagaatctgccgcctgcatcacactttcggcgcctacgccgccgaaatctacgccgccagggggctttacaggatcgacccgatcctcaagcttgcgctcggcggcgtcaggccggtggaatgggcgacagcgcggcgccgctttccggaatgcgagcccctcttcgaggcggccgaagaaatcgggctttccaccgaaggcgtggccttaccgctcccctcgcctgcgggccgcatggcgcttctcgcaatcggtgcaa

SEQ ID NO: 13 - DNA, 407 bp, Sinorhizobium meliloti
tcacatggcctggcgggttgcgcggcgcgtttttgatttgaggatgctctatgaatattacgttgctcgtacagtttctggcgctactggaagagatgaagacgcgcgaggagatcctgcccgagttcgagcgcctgctcgaccgctgcggtttcgacttctacggcatcgtgcgtcagccgaaaccgcatgagaatccgctgagacttcttctggccggacgctggccggagggctggccgcaaatctacatccgcaagaaatacgtcgttatcgatccgaccattcgcttcctcgggcatgcccagcgcggcttccgctggcgcgacacgctcgtggcattccgctcggacccgcaccgcaagcgcatggaaagcatgatggtcgaggcgcgcaatcatggcctc

SEQ ID NO: 14 - DNA, 405 bp, Rhodobacter sphaeroides
catacacaggggggacaagtcaatatggcaaccgaagagcagtctccgggttccggccgtgacgctcagttcgagcgtctgaacgcgaatctcacccgcatcgacgagctgtcgaaacggctgacggccgctctcacgaagcgcaaactgtcggaccccgcgctgcacgggccctcgggcgacgtcttcctgaaggcgatgacggcctacatggccgagatgatgcagaacccggccaagatcctcgagcatcagatcagtttctggggcaagagcctgaaacattacgtcgaggctcagcaccagctggtgaagggcgagctgaagccgccgccggacgtgacgccgaaggaccgccgcttctcgaacccgctctggcagacgcatcccttcttcaactatctc

SEQ ID NO: 15 - DNA, 468 bp, Rhodobacter sphaeroides
gatccgccgctttcgtttccggggtgcgtggtgcgcctcccggaacggcaccggacagtgaaggagccgcagggaagtggcggaggcgttcagaggcgaatacaaccagaaggttgacgccaaggcgcgggtgtcgatcccggcccccttccgtcgtgtcatcgaagcgggcgatcccaaattctccggcggccggtcgagcttcgtgctcgtctatggcggcgaccgctcctacgtcgaatgctacaccatttccgagatggagcggatcgaggaacggatccgcagcctgcccatgggcacgcccaagcggcgctatctcgaacgcaacatgatcaccctcgcgcttaacatggagctcgacgaggacggccggatcgtgctgccgcccaagggccgcgagaagctgggcatctcgcccgacgagctgaagggcggcaccgaagccacctttgcgggcacgctcaa

SEQ ID NO: 16 - DNA, 1806 bp, Rhodobacter sphaeroides
atggcaaccgaagagcagtctccgggttccggccgtgacgctcagttcgagcgtctgaacgcgaatctcacccgcatcgacgagctgtcgaaacggctgacggccgctctcacgaagcgcaaactgtcggaccccgcgctgcacgggccctcgggcgacgtcttcctgaaggcgatgacggcctacatggccgagatgatgcagaacccggccaagatcctcgagcatcagatcagtttctggggcaagagcctgaaacattacgtcgaggctcagcaccagctggtgaagggcgagctgaagccgccgccggacgtgacgccgaaggaccgccgcttctcgaacccgctctggcagacgcatcccttcttcaactatctcaagcagcagtatctgatgaacgccgaggcggtgaatcaggccgtcgaggcgctggagcatatcgagccgtccgacaagaagcgggtcgaatatttctcgcgccagatcgtcgatcttttctcgcccacgaacttcttcggcaccaatcccgacgcgctcgaacgcgccatcgccaccgacggcgagagcctggtgcaggggctggagaatctcgtgcgcgacatcgaggccaacaacggcgatctgctcgtcacgctggccgaccccgaggcctttcaggtggggcagaacctcgccaccaccgaagggtcggtcgtctaccgcaaccgcatgttcgagctgatccagtacaagcccacgaccgagacggtccacgagacgccgctgctgatctttccgccctggatcaacaagttctacatcctcgacctcaagccgcagaattccctgctgaagtggctggtggatcagggcttcacggtcttcgtcgtctcgtgggtgaaccccgacaagagctatgccggcatcggcatggacgactacatccgcgaaggctacatgcgcgccatggccgaggtgcgctcgatcacccggcagaagcagatcaacgcggtaggctattgcatcgcgggcaccacgctcacgctgacgctggcgcacctgcagaaggcgggcgatccgtccgtacgctcggccaccttcttcaccacgctcaccgacttttcggacccgggtgaggtgggggtgttcctcaacgacgatttcgtcgacgggatcgagcggcaggtggcggtggacgggatcctcgacaagaccttcatgtcgcgcaccttcagctatctgcggtcgaacgacctgatctatcagccggcgatcaagagctacatgatgggcgaggcgccgccggccttcgacctgctctactggaacggagacggcaccaacctgccggcgcagatggcggtcgaatacctgcgtggcctgtgccagcaggaccggctggcgggcggcaccttcccggtgctgggctcgcccgtggggctgaaggatgtgacgcttcccgtctgcgccatcgcctgcgagaccgaccatatcgcgccgtggaaaagcagcttcaacggcttccgtcagttcggctcgaccgacaagaccttcattctctctcaatcgggccatgtggcgggcatcgtgaacccgcccagccgcaacaaatacggccattacaccaacgagggcccggccggcacgccggagtcgttccgggagggggccgagttccacgcgggctcctggtggccgcgctggggcgcctggctcgccgagcgatcgggcaagcaggtcccggcgcgccagccgggcgattcgaaacatcccgagctcgcgccggcgcccggatcctatgtggcggcggtgggcggggcttga

SEQ ID NO: 17 - DNA, 1458 bp, Agrobacterium tumefaciens
atgctgttccgcaataagcctgacgcaaaatataaaggcgcatccgtaagattagcctcctatactgttctcggtgtggtggcgacggtgttttcttcttccgtgtttccgcctgtattcacctctcaaacgagccgtgctctgatcaatgcccccattattcccttgacgacgccgatcagcggcgttgtgaaaacattgaacgacaggggtggtgccaccatcgagaacgacaaggtggacaatacaacgctgatcggtctgaaggttcaactggcggcgctcgacaatgagatgcgccagaagaactcgatcgtttcggactatgcctcgcggatcgacgacctgaacagggatctttccagccagcaggcggctttgctgctgcggaccgagtccgatctcgaggctgcagaggcggccttgcagatggttacctattccacgcggatcgcaaaagccgaagcggctcgcaaacaaaaactcgtcgacaagggcgtttttcaaggcataagcgaagacatcgccgatacgatacaacttgaagatacaaaactgaaggcggcacgtgtcgctgtcaacaagctgaacaaggacatgaccttcgcgcggcaggggatttatattggatccgatctgcaatcgctgcagaacctccagcaggaaatccgcaccagaacggctgacctgatgcaggtgcggatgcagatgaccacacttgaaacacggagaagcgaactcgagaccctggcaacgactgaggcctcgcgcatcgacaggttgacgcatgcagatcttgccattccgccgggaacgacgctctacaagccggtggctgccaccgggcgggaagttgtcgccggtgacacgctcgcagaggcactcgattgccgcaacgcgtttgttgtcgctatcttctccgagcgccaggcgcaggcactctccgttggctcgcgtgttaaggtcgatgcggggggctgggcccaggagagcagtggcacggtggaaaggttggtaccgcgcacaactgaacgggtggatcttgattacgctgtcccatttccgccaacagagagacgcgaactttatgcgttcatccgcatggatggtaccgatcagcccgatctttcgcatcagaaatcctgctcggtcggcacatgggtcaatgtgaccctgccaaacgaatggctggacaggacgcgaaactacgttcacgaagcgtccgctgatctcctccaatatgcgaagaactccgcgaaggagattccgtctgtcacgcaggcagccatggcgctccttgaatcgtcgcggaacaggatcttcgcctatatgggaatggaacagccacgccagggacggctgccggagcttgcagcgccgaaccgtcaactggatgacacaaggcatgccgcgaacgggcccgttccccagaccaagatttcgcgaactcaatcctga

SEQ ID NO: 18 - DNA, 1965 bp, Agrobacterium tumefaciens
atgtatttcagtgctgaaggtgacgttcagtcggtgctctatgtgaacctgacgattgcgattggggcgatcctgtttgcccttctcgctgatcccagaaagatggtcgacaggttggccttcagcatcatcatgttgctatcgcttggtgtctatatcgtatggcgggcaacggataccttgccgccgccggaactctccctcgaaacgctctggtgctacacctatttcaccttcgagctgatctcggtgctttatgccatggggtccatcctcatacttcttcgccgaaccgactggtcagccgttgccgatcagggagaggcatatcttgcaggcaacccgcatgcgccgctcgtcgatgtgtttatctgcacttacaacgagccgctgaacgttctcgaaaaatccatcatcgccgcgcaggcgatggattatcctcgactgcgcgtcttcgtctgtgacgacacacgtcgcggggaggtaagaacctattgcgaagccgtaggcgtgaactacgtcacacgtcccgacaacaagcacgccaaggcaggaaatctcaacaatgcgctgctccacaccaatgcgctggaagaggtttccgacttcatcatggtcctcgacgcggattttgccccccaggcaaacttcctgcggcgcgtgacgggtctcttttcggacccgaaggtggctgtcgtccagacgcctcaattctatttcaacagtgatccaattcagcacaatctcggtatagacaagagcttcgtggacgaccagcgggtcttcttcgacgtcttccagccggccaaggatgccgttggttgcgctttttgcgtcggcaccagcttcgtcgtacgccgcgccgcggtaaatggtattggtggtttcccttcggatgcgctttccgaagacatgctgctgacatatcgcctgatggaaaggggatatgtcacgcgctggctgaatgagaagttgagcgttggattgtcggcggaaggtgtacccgaatacatcacccagcgcacccgctggtgtctcggcacgatccagatcgggcttctgcggaccggacctctctggcgtggaaattttacgctgacgcagcggctgcactatctgcatggacttttctgctggctgtcgaagccgtttatcctgtgcctgctgcttgcgccgtccatctattggctgacgggcgtgtcggcgctgcaggtcgatgagctgatgttcatgaagctcggcctgtcatctcttgcgcttttctggacctattccacctggatatccggcaagaggacgcttcctctcttcaccgaagtcacccacgccctgaccgctgtacccattaccatcacgctttttcaggcaatccgtaaaccgttcgggcgcccgttcaaagtcaccgaaaagggaggagaccgatcccaggtccgtgtccacctcccgacggcgatttttttcgctttcgtgaccctgtcttcggccgtctccatcgtgctggctgtctatggtctggatgctccgtccgagctgtcctcgcgggactgcctcaatctgatctggtccgccgtcgcgatggttatcgcattcaccagcttcatttgctgcattgaattgccgcgtttcggcaaggaggaaatgatcggagtggattttcgcgggcagttgcggtccgcatcctcaacgagaccggtgcgtatcaccggcctctcgacggaaaacatcacactggctgcggttccgtcttccagcgatgtaaaggatgttttcgtaccggaggcggggtggatgcggatcagccctgcggagcacgcgcagaactccggaaagttcgatattcatccaagcgacgagcagcgccggtccattttgcgcctgttgtttcgcaaggctcctgaaaatgtcgcggaacagggcgacctgatgaaatccatgcggattcttctcgcacgggcattcgggtga

SEQ ID NO: 19 - DNA, 1266 bp, Agrobacterium tumefaciens
atgagcatccgaaacatgatcgcgacgcttttgatggttttcgcgatgacgggcacggcggcggccgggaaaatagcggatcgtactggtctcgcggcaaagctgtgtgacggccttgcgggcaggatggaccaatcaaccgcaccgtttttgctccgcagcttcgagccggggccgtcacagaagccgctcgatccggcgctgtcaaatacggctttcacctatgataatgcgcttgcctcgattgcgcttttcgcctgtggaaaggatgacaaggcgctgaggatcgtcgaggctctgcgttatgcgcttcagcacgaccggacctatcgcgatgggcgggtgcggaatgcctaccgtgccggtgctgtcgatgttcatcagggctccatcctcctgccgggtttctggaacgagggccgcaaggcttggatggaggacgactatcaggtcggaagcgctaccggaaatcttgcctgggcagcgctggcgtttctcgccgcttttgatcgttcgggagataaatcctatctctccgctgcgtcgtcactcatcgagtggatcaaccagaataccgttggaacaggcggtctcggttttacgggcgggacgttcggtcaggatgctcaacctatacatctcgactggaaatcgacggagcataatcttgacgtctttgccgctgcagcctggctgagcgagatcgaccaggcgaaggactggcgatccgtgcaggaccgggcgtcgtcttttctcaatgccatgtggaacgatggtgagggtcgtttttacgtcggcagtttgcccggtggcgacacgccgaacaccagccagtccggcattgattccgaactttggccgatcatggccgtgccgaaattccgcgcgcgcgcggaccatgttctcgattgggtcgatcgtcattatgccgttgatggcggttttgatttcaacgacgaccgggacggcatatggctggaaggcacggcgcaagctgcgctggcgttcgagattgcggggcatcgcgctcgctcggacgcgcttcttgatacgattggagcggaattgtcgccggagagccttgtctatgccacgtcgggtcccgaattaacgacgggtttgaaaataggcccggattccacatccgcagatttcaaatatttccggttacctcacatcggcgcgacggcatgggggatactcgctgcgaaaggctggaatccgttcgtcaggaggggagtttcaagtatgcacgaggcagaataa

SEQ ID NO: 20 - DNA, 660 bp, Sinorhizobium meliloti
atggccactttggaaggcggcgcatacgacgacgccctgtttggctcccgctttgacgatttcatccgcgcccatgggggtgatgatttcgtcaacggaggcaatggggacgacatcatcttcggcgacgatggtgacgacttgctgttcggcggcaacggaaacgacaccgtgttcggcggcgaaggcaccgacgttctctatggcgaaaatggcaacgatatcctggtcggcggatcgggtgacgacctgatctatggcgataacggcaacgacattctccttgggggcgccggcagcgacttcctcctcggaggcagaggcaacgacgtgttgctcggcggcgccggcaacgacgtcatcgacggcggcgccgggtccgaccttcttgccggcggtcagggcagcgatatcttcgttttcgacggcggtggcggcaacgacgtcatcctcgactttacccccggcgaagacgtcctgcagatatccaagggtatcaacggcctcgacgtcaccgcgcccgaggatctcgcttcgcgtatcactcaggtcggcggcaatgtcgtcatcgacctcggccatggcgacacgctgacgctggtcaatgccgacgccgaagacattcaggcccatcccgaaaactacttcactgtccactga